European Patent Application EP 4 530 355 A2, published April 2, 2025. Title: LENTIVIRAL VECTORS. Applicant: Oxford BioMedica (UK) Limited. The sequence listing filed with the application follows.

SEQUENCE LISTING (264 sequences)

SEQ ID NO: 1 - DNA, 30 bp, synthetic construct
  source 1..30: mol_type = other DNA
ggggcggcgactggtgagtacgccaaaaat

SEQ ID NO: 2 - DNA, 30 bp, synthetic construct
  source 1..30: mol_type = other DNA
ggggcggcgactgcagacaacgccaaaaat

SEQ ID NO: 3 - DNA, 30 bp, synthetic construct
  source 1..30: mol_type = other DNA
ggggcggcgagtggagactacgccaaaaat

SEQ ID NO: 4 - DNA, 32 bp, synthetic construct
  source 1..32: mol_type = other DNA
ggggaaggcaacagataaatatgccttaaaat

SEQ ID NO: 5 - DNA, 19 bp, synthetic construct
  source 1..19: mol_type = other DNA
ggcgactggtgagtacgcc

SEQ ID NO: 6 - DNA, 19 bp, synthetic construct
  source 1..19: mol_type = other DNA
ggcgactgcagacaacgcc

SEQ ID NO: 7 - DNA, 19 bp, synthetic construct
  source 1..19: mol_type = other DNA
ggcgagtggagactacgcc

SEQ ID NO: 8 - DNA, 23 bp, synthetic construct
  source 1..23: mol_type = other DNA
aaggcaacagataaatatgcctt

SEQ ID NO: 9 - DNA, 339 bp, synthetic construct
  source 1..339: mol_type = other DNA
atgggtgcgagagcgtcagtattaagcgggggagaattagatcgcgatgggaaaaaattcggttaaggccagggggaaagaaaaaatataaattaaaacatatagtatgggcaagcagggagctagaacgattcgcagttaatcctggcctgttagaaacatcagaaggctgtagacaaatactgggacagctacaaccatcccttcagacaggatcagaagaacttagatcattatataatacagtagcaaccctctattgtgtgcatcaaaggatagagataaaagacaccaaggaagctttagacaagatagagggagagcaaaacaaaagtaaga

SEQ ID NO: 10 - DNA, 81 bp, synthetic construct
  source 1..81: mol_type = other DNA
atgggtgcgagagcgtcagtattaagcgggggagaattagatcgcgatgggaaaaaattcggttaaggccagggggaaaga

SEQ ID NO: 11 - DNA, 341 bp, synthetic construct
  source 1..341: mol_type = other DNA
acgggtgcgagagcgtcagtattaagcgggggagaattagatcgcgattgggaaaaaattcggttaaggccagggggaaagaaaaaatataaattaaaacatatagtattgggcaagcagggagctagaacgattcgcagttaatcctggcctgttagaaacatcagaaggctgtagacaaatactgggacagctacaaccatcccttcagacaggatcagaagaacttagatcattatataatacagtagcaaccctctattgtgtgcatcaaaggatagagataaaagacaccaaggaagctttagacaagatagagggagagcaaaacaaaagtaaga

SEQ ID NO: 12 - DNA, 82 bp, synthetic construct
  source 1..82: mol_type = other DNA
acgggtgcgagagcgtcagtattaagcgggggagaattagatcgcgattgggaaaaaattcggttaaggccagggggaaaga

SEQ ID NO: 13 - DNA, 255 bp, synthetic construct
  source 1..255: mol_type = other DNA
aaaaatataaattaaaacatatagtatgggcaagcagggagctagaacgattcgcagttaatcctggcctgttagaaacatcagaaggctgtagacaaatactgggacagctacaaccatcccttcagacaggatcagaagaacttagatcattatataatacagtagcaaccctctattgtgtgcatcaaaggatagagataaaagacaccaaggaagctttagacaagatagagggagagcaaaacaaaagta

SEQ ID NO: 14 - DNA, 234 bp, synthetic construct
  source 1..234: mol_type = other DNA
aggagctttgttccttgggttcttgggagcagcaggaagcactatgggcgcagcgtcaatgacgctgacggtacaggccagacaattattgtctggtatagtgcagcagcagaacaatttgctgagggctattgaggcgcaacagcatctgttgcaactcacagtctggggcatcaagcagctccaggcaagaatcctggctgtggaaagatacctaaaggatcaacagctcct

SEQ ID NO: 15 - DNA, 783 bp, synthetic construct
  source 1..783: mol_type = other DNA
tgatcttcagacctggaggaggagatatgagggacaattggagaagtgaattatataaatataaagtagtaaaaattgaaccattaggagtagcacccaccaaggcaaagagaagagtggtgcagagagaaaaaagagcagtgggaataggagctttgttccttgggttcttgggagcagcaggaagcactatgggcgcagcgtcaatgacgctgacggtacaggccagacaattattgtctggtatagtgcagcagcagaacaatttgctgagggctattgaggcgcaacagcatctgttgcaactcacagtctggggcatcaagcagctccaggcaagaatcctggctgtggaaagatacctaaaggatcaacagctcctggggatttggggttgctctggaaaactcatttgcaccactgctgtgccttggaatgctagttggagtaataaatctctggaacagatttggaatcacacgacctggatggagtgggacagagaaattaacaattacacaagcttaatacactccttaattgaagaatcgcaaaaccagcaagaaaagaatgaacaagaattattggaattagataaatgggcaagtttgtggaattggtttaacataacaaattggctgtggtatataaaattattcataatgatagtaggaggcttggtaggtttaagaatagtttttgctgtactttctatagtgaatagagttaggcagggatattcaccattatcgtttcagacccacctcccaaccccgaggggac

SEQ ID NO: 16 - DNA, 236 bp, synthetic construct
  source 1..236: mol_type = other DNA
aggagctttgttccttgggttcttgggagcagcaggaagcactattgggcgcagcgtcaattgacgctgacggtacaggccagacaattattgtctggtatagtgcagcagcagaacaatttgctgagggctattgaggcgcaacagcatctgttgcaactcacagtctggggcatcaagcagctccaggcaagaatcctggctgtggaaagatacctaaaggatcaacagctcct

SEQ ID NO: 17 - DNA, 789 bp, synthetic construct
  source 1..789: mol_type = other DNA
tgatcttcagacctggaggaggagatattgagggacaattggagaagtgaattatataaatataaagtagtaaaaattgaaccattaggagtagcacccaccaaggcaaagagaagagtggtgcagagagaaaaaagagcagtgggaataggagctttgttccttgggttcttgggagcagcaggaagcactattgggcgcagcgtcaattgacgctgacggtacaggccagacaattattgtctggtatagtgcagcagcagaacaatttgctgagggctattgaggcgcaacagcatctgttgcaactcacagtctggggcatcaagcagctccaggcaagaatcctggctgtggaaagatacctaaaggatcaacagctcctggggatttggggttgctctggaaaactcatttgcaccactgctgtgccttggaattgctagttggagtaataaatctctggaacagatttggaatcacacgacctggattggagtgggacagagaaattaacaattacacaagcttaatacactccttaattgaagaatcgcaaaaccagcaagaaaagaatgaacaagaattattggaattagataaatgggcaagtttgtggaattggtttaacataacaaattggctgtggtatataaaattattcataattgatagtaggaggcttggtaggtttaagaatagtttttgctgtactttctatagtgaatagagttaggcagggatattcaccattatcgtttcagacccacctcccaaccccgaggggac

SEQ ID NO: 18 - DNA, 791 bp, synthetic construct
  source 1..791: mol_type = other DNA
tgatcttcagacctggaggaggagatattgagggacaattggagaagtgaattatataaatataaagtagtaaaaattgaaccattaggagtagcacccaccaaggcaaagagaagagtggtgcagagagaaaaaagagcagtgggaataggagctttgttccttgggttcttgggagcagcaggaagcactattgggcgcagcgtcaattgacgctgacggtacaggccagacaattattgtctggtatagtgcagcagcagaacaatttgctgagggctattgaggcgcaacagcatctgttgcaactcacagtctggggcatcaagcagctccaggcaagaatcctggctgtggaaagatacctaaaggatcaacagctcctggggatttggggttgctctggaaaactcatttgcaccactgctgtgccttggaattgctagttggagtaataaatctctggaacagatttggaatcacacgacctggattggagtgggacagagaaattaacaattacacaagcttaatacactccttaattgaagaatcgcaaaaccagcaagaaaagaattgaacaagaattattggaattagataaattgggcaagtttgtggaattggtttaacataacaaattggctgtggtatataaaattattcataattgatagtaggaggcttggtaggtttaagaatagtttttgctgtactttctatagtgaatagagttaggcagggatattcaccattatcgtttcagacccacctcccaaccccgaggggac

SEQ ID NO: 19 - DNA, 585 bp, synthetic construct
  source 1..585: mol_type = other DNA
aatcaacctctggattacaaaatttgtgaaagattgactggtattcttaactatgttgctccttttacgctatgtggatacgctgctttaatgcctttgtatcatgctattgcttcccgtatggctttcattttctcctccttgtataaatcctggttgctgtctctttatgaggagttgtggcccgttgtcaggcaacgtggcgtggtgtgcactgtgtttgctgacgcaacccccactggttggggcattgccaccacctgtcagctcctttccgggactttcgctttccccctccctattgccacggcggaactcatcgccgcctgccttgcccgctgctggacaggggctcggctgttgggcactgacaattccgtggtgttgtcggggaagctgacgtcctttccatggctgctcgcctgtgttgccacctggattctgcgcgggacgtccttctgctacgtcccttcggccctcaatccagcggaccttccttcccgcggcctgctgccggctctgcggcctcttccgcgtcttcgccttcgccctcagacgagtcggatctccctttgggccgcctcc

SEQ ID NO: 20 - DNA, 585 bp, synthetic construct
  source 1..585: mol_type = other DNA
aatcaacctctggattacaaaatttgtgaaagattgactggtattcttaactatgttgctccttttacgctatgtggatacgctgctttaatgcctttgtatcatgctattgcttcccgtatggctttcattttctcctccttgtataaatcctggttgctgtctctttatgaggagttgtggcccgttgtcaggcaacgtggcgtggtgtgcactgtgtttgctgacgcaacccccactggttggggcattgccaccacctgtcagctcctttccgggactttcgctttccccctccctattgccacggcggaactcatcgccgcctgccttgcccgctgctggacaggggctcggctgttgggcactgacaattccgtggtgttgtcggggaaatcatcgtcctttccttggctgctcgcctgtgttgccacctggattctgcgcgggacgtccttctgctacgtcccttcggccctcaatccagcggaccttccttcccgcggcctgctgccggctctgcggcctcttccgcgtcttcgccttcgccctcagacgagtcggatctccctttgggccgcctcc

SEQ ID NO: 21 - DNA, 482 bp, synthetic construct
  source 1..482: mol_type = other DNA
atgctattgcttcccgtatggctttcattttctcctccttgtataaatcctggttgctgtctctttatgaggagttgtggcccgttgtcaggcaacgtggcgtggtgtgcactgtgtttgctgacgcaacccccactggttggggcattgccaccacctgtcagctcctttccgggactttcgctttccccctccctattgccacggcggaactcatcgccgcctgccttgcccgctgctggacaggggctcggctgttgggcactgacaattccgtggtgttgtcggggaaatcatcgtcctttccttggctgctcgcctgtgttgccacctggattctgcgcgggacgtccttctgctacgtcccttcggccctcaatccagcggaccttccttcccgcggcctgctgccggctctgcggcctcttccgcgtcttcgccttcgccctcagacgagtcggatctccctttgggccgcctcc

SEQ ID NO: 22 - DNA, 587 bp, synthetic construct
  source 1..587: mol_type = other DNA
aatcaacctctggattacaaaatttgtgaaagattgactggtattcttaactatgttgctccttttacgctatgtggatacgctgctttaatgcctttgtatcattgctattgcttcccgtatggctttcattttctcctccttgtataaatcctggttgctgtctctttattgaggagttgtggcccgttgtcaggcaacgtggcgtggtgtgcactgtgtttgctgacgcaacccccactggttggggcattgccaccacctgtcagctcctttccgggactttcgctttccccctccctattgccacggcggaactcatcgccgcctgccttgcccgctgctggacaggggctcggctgttgggcactgacaattccgtggtgttgtcggggaaatcatcgtcctttccttggctgctcgcctgtgttgccacctggattctgcgcgggacgtccttctgctacgtcccttcggccctcaatccagcggaccttccttcccgcggcctgctgccggctctgcggcctcttccgcgtcttcgccttcgccctcagacgagtcggatctccctttgggccgcctcc

SEQ ID NO: 23 - DNA, 591 bp, synthetic construct
  source 1..591: mol_type = other DNA
aatcaacctctggattacaaaatttgtgaaagattgactggtattcttaactattgttgctccttttacgctattgtggatacgctgctttaattgcctttgtatcattgctattgcttcccgtattggctttcattttctcctccttgtataaatcctggttgctgtctctttattgaggagttgtggcccgttgtcaggcaacgtggcgtggtgtgcactgtgtttgctgacgcaacccccactggttggggcattgccaccacctgtcagctcctttccgggactttcgctttccccctccctattgccacggcggaactcatcgccgcctgccttgcccgctgctggacaggggctcggctgttgggcactgacaattccgtggtgttgtcggggaaatcatcgtcctttccttggctgctcgcctgtgttgccacctggattctgcgcgggacgtccttctgctacgtcccttcggccctcaatccagcggaccttccttcccgcggcctgctgccggctctgcggcctcttccgcgtcttcgccttcgccctcagacgagtcggatctccctttgggccgcctcc

SEQ ID NO: 24 - DNA, 97 bp, synthetic construct
  source 1..97: mol_type = other DNA
gggtctctctggttagaccagatctgagcctgggagctctctggctaactagggaacccactgcttaagcctcaataaagcttgccttgagtgcttc

SEQ ID NO: 25 - DNA, 60 bp, synthetic construct
  source 1..60: mol_type = other DNA
gggtctctctggttagaccagatctgagcctgggagctctctggctaactagggaaccca

SEQ ID NO: 26 - DNA, 25 bp, synthetic construct
  source 1..25: mol_type = other DNA
gggtctctctggttagaccagatca

SEQ ID NO: 27 - DNA, 20 bp, synthetic construct
  source 1..20: mol_type = other DNA
gggtctctctggttagacca

SEQ ID NO: 28 - DNA, 46 bp, synthetic construct
  source 1..46: mol_type = other DNA
gggtctctctggttagaccacacacatggtctaaccagagagaccc

SEQ ID NO: 29 - DNA, 18 bp, synthetic construct
  source 1..18: mol_type = other DNA
gtctctctggttagacca

SEQ ID NO: 30 - DNA, 16 bp, synthetic construct
  source 1..16: mol_type = other DNA
gggtctctctggttag

SEQ ID NO: 31 - DNA, 14 bp, synthetic construct
  source 1..14: mol_type = other DNA
gtctctctggttag

SEQ ID NO: 32 - DNA, 14 bp, synthetic construct
  source 1..14: mol_type = other DNA
gggtctctctggtt

SEQ ID NO: 33 - DNA, 12 bp, synthetic construct
  source 1..12: mol_type = other DNA
gtctctctggtt

SEQ ID NO: 34 - DNA, 12 bp, synthetic construct
  source 1..12: mol_type = other DNA
gggtctctctgg

SEQ ID NO: 35 - DNA, 10 bp, synthetic construct
  source 1..10: mol_type = other DNA
gtctctctgg

SEQ ID NO: 36 - DNA, 10 bp, synthetic construct
  source 1..10: mol_type = other DNA
gggtctctct

SEQ ID NO: 37 - DNA, 37 bp, synthetic construct
  source 1..37: mol_type = other DNA
aataaagggtctctctggttagaccacaagttaacaa

SEQ ID NO: 38 - DNA, 35 bp, synthetic construct
  source 1..35: mol_type = other DNA
aataaagggtctctctggttagaccaagttaacaa

SEQ ID NO: 39 - DNA, 63 bp, synthetic construct
  source 1..63: mol_type = other DNA
aataaagggtctctctggttagaccacacacatggtctaaccagagagaccccaagttaacaa

SEQ ID NO: 40 - DNA, 35 bp, synthetic construct
  source 1..35: mol_type = other DNA
aataaagtctctctggttagaccacaagttaacaa

SEQ ID NO: 41 - DNA, 33 bp, synthetic construct
  source 1..33: mol_type = other DNA
aataaagggtctctctggttagcaagttaacaa

SEQ ID NO: 42 - DNA, 31 bp, synthetic construct
  source 1..31: mol_type = other DNA
aataaagtctctctggttagcaagttaacaa

SEQ ID NO: 43 - DNA, 31 bp, synthetic construct
  source 1..31: mol_type = other DNA
aataaagggtctctctggttcaagttaacaa

SEQ ID NO: 44 - DNA, 29 bp, synthetic construct
  source 1..29: mol_type = other DNA
aataaagtctctctggttcaagttaacaa

SEQ ID NO: 45 - DNA, 29 bp, synthetic construct
  source 1..29: mol_type = other DNA
aataaagggtctctctggcaagttaacaa

SEQ ID NO: 46 - DNA, 27 bp, synthetic construct
  source 1..27: mol_type = other DNA
aataaagtctctctggcaagttaacaa

SEQ ID NO: 47 - DNA, 27 bp, synthetic construct
  source 1..27: mol_type = other DNA
aataaagggtctctctcaagttaacaa

SEQ ID NO: 48 - DNA, 25 bp, synthetic construct
  source 1..25: mol_type = other DNA
aataaagtctctctcaagttaacaa

SEQ ID NO: 49 - DNA, 37 bp, synthetic construct
  source 1..37: mol_type = other DNA
aataaagggtctctctggttagaccagatcattgcaa

SEQ ID NO: 50 - DNA, 34 bp, synthetic construct
  source 1..34: mol_type = other DNA
aataaagggtctctctggttagaccacattgcaa

SEQ ID NO: 51 - DNA, 32 bp, synthetic construct
  source 1..32: mol_type = other DNA
aataaagggtctctctggttagaccattgcaa

SEQ ID NO: 52 - DNA, 30 bp, synthetic construct
  source 1..30: mol_type = other DNA
aataaagggtctctctggttagcattgcaa

SEQ ID NO: 53 - DNA, 28 bp, synthetic construct
  source 1..28: mol_type = other DNA
aataaagggtctctctggttcattgcaa

SEQ ID NO: 54 - DNA, 26 bp, synthetic construct
  source 1..26: mol_type = other DNA
aataaagggtctctctggcattgcaa

SEQ ID NO: 55 - DNA, 258 bp, synthetic construct
  source 1..258: mol_type = other DNA
aaaagaaaaggggggactggaagggctaattcactcccaacgaagacaagatactagtaaaaaaatgctttatttgtgaaatttgtgatgctattgctttatttgtaaccattataagctgcaataaagggtctctctggttagaccagatctgagcctgggagctctctggctaactagggaacccacaagttaacaacaacaattgcattcattttatgtttcaggttcagggggaggtgtgggaggttttttaaa

SEQ ID NO: 56 - DNA, 244 bp, synthetic construct
  source 1..244: mol_type = other DNA
aaaagaaaaggggggactggaagggctaattcactcccaacgaagacaagatactagtaaaaaaatgctttatttgtgaaatttgtgatgctattgctttatttgtaaccattataagctgcaataaagggtctctctggttagaccacacacatggtctaaccagagagaccccaagttaacaacaacaattgcattcattttatgtttcaggttcagggggaggtgtgggaggttttttaaa

SEQ ID NO: 57 - DNA, 218 bp, synthetic construct
  source 1..218: mol_type = other DNA
aaaagaaaaggggggactggaagggctaattcactcccaacgaagacaagatactagtaaaaaaatgctttatttgtgaaatttgtgatgctattgctttatttgtaaccattataagctgcaataaagggtctctctggttagaccacaagttaacaacaacaattgcattcattttatgtttcaggttcagggggaggtgtgggaggttttttaaa

SEQ ID NO: 58 - DNA, 364 bp, synthetic construct
  source 1..364: mol_type = other DNA
aaaagaaaaggggggactggaagggctaattcactcccaacgaagacaagatactagtgaattcactcctcaggtgcaggctgcctatcagaaggtggtggctggtgtggccaatgccctggctcacaaataccactgagatctttttccctctgccaaaaattatggggacatcatgaagccccttgagcatctgacttctggctaataaagggtctctctggttagaccagatcattgcaatagtgtgttggaattttttgtgtctctcactcggaaggacatatgggagggcaaatcatttaaaacatcagaatgagtatttggtttagagtttggcaacatatgcccatatgctggctgc

SEQ ID NO: 59 - DNA, 273 bp, synthetic construct
  source 1..273: mol_type = other DNA
aaaagaaaaggggggactggaagggctaattcactcccaacgaagacaagatactagtcagacatgataagatacattgatgagtttggacaaaccacaactagaatgcagtgaaaaaaatgctttatttgtgaaatttgtgatgctattgctttatttgtaaccattataagctgcaataaagggtctctctggttagaccacaagttaacaacaacaattgcattcattttatgtttcaggttcagggggaggtgtgggaggttttttaaa

SEQ ID NO: 60 - DNA, 250 bp, synthetic construct
  source 1..250: mol_type = other DNA
aaaagaaaaggggggactggaagggctaattcactcccaacgaagacaagatactagtcacacaaaaaaccaacacacagatgtaatgaaaataaagatctttatttgtgaaatttgtgatgctattgctttatttgtaaccattataagctgcaataaagggtctctctggttagaccacaagttaacaacaacaattgcattcattttatgtttcaggttcagggggaggtgtgggaggttttttaaa

SEQ ID NO: 61 - DNA, 54 bp, synthetic construct
  source 1..54: mol_type = other DNA
gggtctctctggttagaccacacattggtgtgcacctggctaactagggaaccc

SEQ ID NO: 62 - DNA, 59 bp, synthetic construct
  source 1..59: mol_type = other DNA
gggtctctctggttagaccacacattcgtgtgtttgtgtctgttctaactagggaaccc

SEQ ID NO: 63 - DNA, 60 bp, synthetic construct
  source 1..60: mol_type = other DNA
gggtctctctggttagaccacacacttcgtgtgtttgtgtctgttctaactagggaaccc

SEQ ID NO: 64 - DNA, 61 bp, synthetic construct
  source 1..61: mol_type = other DNA
gggtctctctggttagaccacacacattcgtgtgtttgtgtctgttctaactagggaaccc

SEQ ID NO: 65 - DNA, 62 bp, synthetic construct
  source 1..62: mol_type = other DNA
gggtctctctggttagaccacacacagttcgtgtgtttgtgtctgttctaactagggaaccc

SEQ ID NO: 66 - DNA, 62 bp, synthetic construct
  source 1..62: mol_type = other DNA
gggtctctctggttagaccacacacaattcgtgtgtttgtgtctgttctaactagggaaccc

SEQ ID NO: 67 - DNA, 63 bp, synthetic construct
  source 1..63: mol_type = other DNA
gggtctctctggttagaccacacacagattcgtgtgtttgtgtctgttctaactagggaaccc

SEQ ID NO: 68 - DNA, 66 bp, synthetic construct
  source 1..66: mol_type = other DNA
gggtctctctggttagaccacacattccagattcgtgtgtttgtgtctgttctaactagggaaccc

SEQ ID NO: 69 - DNA, 56 bp, synthetic construct
  source 1..56: mol_type = other DNA
gggtctctctggttagaccacacatggtgtgcacctgggttctaactagggaaccc

SEQ ID NO: 70 - DNA, 58 bp, synthetic construct
  source 1..58: mol_type = other DNA
gggtctctctggttagaccacacattggtgtgcacctgtggttctaactagggaaccc

SEQ ID NO: 71 - DNA, 64 bp, synthetic construct
  source 1..64: mol_type = other DNA
gggtctctctggttagaccacacatgtctcgtgtgtttgtgtctgttcgctaactagggaaccc

SEQ ID NO: 72 - DNA, 56 bp, synthetic construct
  source 1..56: mol_type = other DNA
gggtctctctggttacaccacaatttggtgtgcacctgggtttaactagggaaccc

SEQ ID NO: 73 - DNA, 64 bp, synthetic construct
  source 1..64: mol_type = other DNA
gggtctctctggttagaccggcgcagcgtcattggtgtgcacctgggttctaactagggaaccc

SEQ ID NO: 74 - DNA, 68 bp, synthetic construct
  source 1..68: mol_type = other DNA
gggtctctctggttagacgcacaacacaaaaccgtgtgttggttttttgtgtgctaactagggaaccc

SEQ ID NO: 75 - DNA, 15 bp, synthetic construct
  source 1..15: mol_type = other DNA
ttggtgtgcacctgg

SEQ ID NO: 76 - DNA, 17 bp, synthetic construct
  source 1..17: mol_type = other DNA
gtgtgtttgtgtctgtt

SEQ ID NO: 77 - DNA, 17 bp, synthetic construct
  source 1..17: mol_type = other DNA
tggtgtgcacctgggtt

SEQ ID NO: 78 - DNA, 19 bp, synthetic construct
  source 1..19: mol_type = other DNA
ttggtgtgcacctgtggtt

SEQ ID NO: 79 - DNA, 19 bp, synthetic construct
  source 1..19: mol_type = other DNA
gtgtgtttgtgtctgttcg

SEQ ID NO: 80 - DNA, 20 bp, synthetic construct
  source 1..20: mol_type = other DNA
tttggtgtgcacctgggttt

SEQ ID NO: 81 - DNA, 18 bp, synthetic construct
  source 1..18: mol_type = other DNA
ttggtgtgcacctgggtt

SEQ ID NO: 82 - DNA, 18 bp, synthetic construct
  source 1..18: mol_type = other DNA
gtgtgttggttttttgtg

SEQ ID NO: 83 - DNA, 37 bp, synthetic construct
  source 1..37: mol_type = other DNA
atttgtgaaatttgtgatgctattgctttatttgtaa

SEQ ID NO: 84 - DNA, 523 bp, synthetic construct
  source 1..523: mol_type = other DNA
cgttacataacttacggtaaatggcccgcctggctgaccgcccaacgacccccgcccattgacgtcaataatgacgtatgttcccatagtaacgccaatagggactttccattgacgtcaatgggtggagtatttacggtaaactgcccacttggcagtacatcaagtgtatcatatgccaagtacgccccctattgacgtcaatgacggtaaatggcccgcctggcattatgcccagtacatgaccttatgggactttcctacttggcagtacatctacgtattagtcatcgctattaccatggtgatgcggttttggcagtacatcaatgggcgtggatagcggtttgactcacggggatttccaagtctccaccccattgacgtcaatgggagtttgttttggcaccaaaatcaacgggacttccgccccattgacgcaaatgggcggtaggcgtgtacggtgggaggtctatataagtgcctagctcgatacaataaacgtctctctggttagaccaca

SEQ ID NO: 85 - DNA, 523 bp, synthetic construct
  source 1..523: mol_type = other DNA
cgttacataacttacggtaaatggcccgcctggctgaccgcccaacgacccccgcccattgacgtcaataatgacgtatgttcccatagtaacgccaatagggactttccattgacgtcaatgggtggagtatttacggtaaactgcccacttggcagtacatcaagtgtatcatatgccaagtacgccccctattgacgtcaatgacggtaaatggcccgcctggcattatgcccagtacatgaccttatgggactttcctacttggcagtacatctacgtattagtcatcgctattaccatggtgatgcggttttggcagtacatcaatgggcgtggatagcggtttgactcacggggatttccaagtctccaccccattgacgtcaatgggagtttgttttggcaccaaaatcaacgggacttccgccccattgacgcaaatgggcggtaggcgtgtacggtggatattgtatttaagtgcctagctcgatacaataaacgtctctctggttagaccaca

SEQ ID NO: 86 - DNA, 207 bp, synthetic construct
  source 1..207: mol_type = other DNA
ttcgagcagacatgataagatacattgatgagtttggacaaaccacaactagaatgcagtgaaaaaaatgctttatttgtgaaatttgtgatgctattgctttatttgtaaccattataagctgcaataaacaagttaacaacaacaattgcattcattttatgtttcaggttcagggggagatgtgggaggttttttaaagcaagt

SEQ ID NO: 87 - DNA, 523 bp, synthetic construct
  source 1..523: mol_type = other DNA
gaattcactcctcaggtgcaggctgcctatcagaaggtggtggctggtgtggccaatgccctggctcacaaataccactgagatctttttccctctgccaaaaattatggggacatcatgaagccccttgagcatctgacttctggctaataaaggaaatttattttcattgcaatagtgtgttggaattttttgtgtctctcactcggaaggacatatgggagggcaaatcatttaaaacatcagaatgagtatttggtttagagtttggcaacatatgcccatatgctggctgccatgaacaaaggttggctataaagaggtcatcagtatatgaaacagccccctgctgtccattccttattccatagaaaagccttgacttgaggttagattttttttatattttgttttgtgttatttttttctttaacatccctaaaattttccttacatgttttactagccagatttttcctcctctcctgactactcccagtcatagctgtccctcttctcttat

SEQ ID NO: 88 - DNA, 225 bp, synthetic construct
  source 1..225: mol_type = other DNA
ctgtgccttctagttgccagccatctgttgtttgcccctcccccgtgccttccttgaccctggaaggtgccactcccactgtcctttcctaataaaatgaggaaattgcatcgcattgtctgagtaggtgtcattctattctggggggtggggtggggcaggacagcaagggggaggattgggaagacaatagcaggcatgctggggatgcggtgggctctatgg

SEQ ID NO: 89 - DNA, 225 bp, synthetic construct
  source 1..225: mol_type = other DNA
ctagctgcccgggtggcatccctgtgacccctccccagtgcctctcctggccctggaagttgccactccagtgcccaccagccttgtcctaataaaattaagttgcatcattttgtctgactaggtgtccttctataatattatggggtggaggggggtggtatggagcaaggggcaagttgggaagacaacctgtagggcctgcggggtctattgggaaccaag

SEQ ID NO: 90 - DNA, 351 bp, synthetic construct
  source 1..351: mol_type = other DNA
ggagctttgttccttgggttcttgggagcagcaggaagcactatgggcgcagcgtcaatgacgctgacggtacaggccagacaattattgtctggtatagtgcagcagcagaacaatttgctgagggctattgaggcgcaacagcatctgttgcaactcacagtctggggcatcaagcagctccaggcaagaatcctggctgtggaaagatacctaaaggatcaacagctcctggggatttggggttgctctggaaaactcatttgcaccactgctgtgccttggaatgctagttggagtaataaatctctggaacagatttggaatcacacgacctggatggagtgggac

SEQ ID NO: 91 - DNA, 355 bp, synthetic construct
  source 1..355: mol_type = other DNA
ggagctttgttccttgggttcttgggagcagcaggaagcactattgggcgcagcgtcaattgacgctgacggtacaggccagacaattattgtctggtatagtgcagcagcagaacaatttgctgagggctattgaggcgcaacagcatctgttgcaactcacagtctggggcatcaagcagctccaggcaagaatcctggctgtggaaagatacctaaaggatcaacagctcctggggatttggggttgctctggaaaactcatttgcaccactgctgtgccttggaattgctagttggagtaataaatctctggaacagatttggaatcacacgacctggattggagtgggac

SEQ ID NO: 92 - DNA, 10 bp, synthetic construct
  source 1..10: mol_type = other DNA
bmwghwssws

SEQ ID NO: 93 - DNA, 34 bp, synthetic construct
  source 1..34: mol_type = other DNA
aaaagaaaaggggggactggaagggctaattcac

SEQ ID NO: 94 - DNA, 81 bp, synthetic construct
  source 1..81: mol_type = other DNA
ccaatgacttacaaggcagctgtagatcttagccactttttaaaagaaaaggggggactggaagggctaattcactcccaa

SEQ ID NO: 95 - DNA, 198 bp, synthetic construct
  source 1..198: mol_type = other DNA
ctcggcaacggcctggtctgtgccaagtgtttgctgacgcaacccccactggttggggcttggccataggccatcagcgcatgcgtggaacctttgtgtctcctctgccgatccatactgcggaactcctagccgcttgttttgctcgcagcaggtctggagcaaacctcatcgggaccgacaattctgtcgtactct

SEQ ID NO: 96 - DNA, 10 bp, synthetic construct
  source 1..10: mol_type = other DNA
cmaghwsstg

SEQ ID NO: 97 - DNA, 10 bp, synthetic construct
  source 1..10: mol_type = other DNA
ccagttcctg

SEQ ID NO: 98 - DNA, 10 bp, synthetic construct
  source 1..10: mol_type = other DNA
ccagatcctg

SEQ ID NO: 99 - DNA, 10 bp, synthetic construct
  source 1..10: mol_type = other DNA
ccagttcctc

SEQ ID NO: 100 - DNA, 10 bp, synthetic construct
  source 1..10: mol_type = other DNA
tcagatcctg

SEQ ID NO: 101 - DNA, 10 bp, synthetic construct
  source 1..10: mol_type = other DNA
ccagatggtg

SEQ ID NO: 102 - DNA, 10 bp, synthetic construct
  source 1..10: mol_type = other DNA
ccagttccag

SEQ ID NO: 103 - DNA, 10 bp, synthetic construct
  source 1..10: mol_type = other DNA
ccagcagctg

SEQ ID NO: 104 - DNA, 10 bp, synthetic construct
  source 1..10: mol_type = other DNA
caagctcctg

SEQ ID NO: 105 - DNA, 10 bp, synthetic construct
  source 1..10: mol_type = other DNA
caagatcctg

SEQ ID NO: 106 - DNA, 10 bp, synthetic construct
  source 1..10: mol_type = other DNA
cctgaacctg

SEQ ID NO: 107 - DNA, 10 bp, synthetic construct
  source 1..10: mol_type = other DNA
caagaacgtg

SEQ ID NO: 108 - DNA, 23 bp, synthetic construct
  source 1..23: mol_type = other DNA
tcctcgtaggctggtcctgggga

SEQ ID NO: 109 - DNA, 20 bp, synthetic construct
  source 1..20: mol_type = other DNA
gcccgctgctggacaggggc

SEQ ID NO: 110 - DNA, 72 bp, synthetic construct
  source 1..72: mol_type = other DNA
tgccgtcgccaccgcgttatccgttcctcgtaggctggtcctggggaacgggtcggcggccggtcggcttct

SEQ ID NO: 111 - DNA, 90 bp, synthetic construct
  source 1..90: mol_type = other DNA
ctattgccacggcggaactcatcgccgcctgccttgcccgctgctggacaggggctcggctgttgggcactgacaattccgtggtgttgt

SEQ ID NO: 112 - DNA, 160 bp, synthetic construct
  source 1..160: mol_type = other DNA
caggaactggcaggaactggcaggaactggcaggaactggcaggaactggcaggaactggcaggaactggcaggaactggcaggaactggcaggaactggcaggaactggcaggaactggcaggaactggcaggaactggcaggaactggcaggaactgg

SEQ ID NO: 113 - DNA, 158 bp, synthetic construct
  source 1..158: mol_type = other DNA
aatcaacctctggattacaaaatttgtgaaagattgactggtattcttaactatgttgctccttttacgctatgtggatacgctgctttaatgcctttgtatcatgctattgcttcccgtatggctttcattttctcctccttgtataaatcctggtt

SEQ ID NO: 114 - DNA, 257 bp, synthetic construct
  source 1..257: mol_type = other DNA
gctgtctctttatgaggagttgtggcccgttgtcaggcaacgtggcgtggtgtgcactgtgtttgctgacgcaacccccactggttggggcattgccaccacctgtcagctcctttccgggactttcgctttccccctccctattgccacggcggaactcatcgccgcctgccttgcccgctgctggacaggggctcggctgttgggcactgacaattccgtggtgttgtcggggaagctgacgtcctttccatggc

SEQ ID NO: 115 - DNA, 177 bp, synthetic construct
  source 1..177: mol_type = other DNA
tgctcgcctgtgttgccacctggattctgcgcgggacgtccttctgctacgtcccttcggccctcaatccagcggaccttccttcccgcggcctgctgccggctctgcggcctcttccgcgtcttcgccttcgccctcagacgagtcggatctccctttgggccgcctccccgcctg

SEQ ID NO: 116 - DNA, 20 bp, synthetic construct
  source 1..20: mol_type = other DNA
ccagttcctgccagttcctg

SEQ ID NO: 117 - DNA, 30 bp, synthetic construct
  source 1..30: mol_type = other DNA
ccagttcctgccagttcctgccagttcctg

SEQ ID NO: 118 - DNA, 24 bp, synthetic construct
  source 1..24: mol_type = other DNA
ttgctcgcagcaggtctggagcaa

SEQ ID NO: 119 - RNA, 11 nt, synthetic construct
  source 1..11: mol_type = other RNA
maggtaagtat

SEQ ID NO: 120 - DNA, 25 bp, synthetic construct
  source 1..25: mol_type = other DNA
gaacacaggtaagtgccgtgtgtgg

SEQ ID NO: 121 - DNA, 25 bp, synthetic construct
  source 1..25: mol_type = other DNA
gtcacttggtgagtagcgggctgct

SEQ ID NO: 122 - DNA, 25 bp, synthetic construct
  source 1..25: mol_type = other DNA
gggcgggagtcgctgcgttgccttc

SEQ ID NO: 123 - DNA, 25 bp, synthetic construct
  source 1..25: mol_type = other DNA
ctgggcaggtaagtatcaaggttac

SEQ ID NO: 124 - DNA, 19 bp, synthetic construct
  source 1..19: mol_type = other DNA
ggcgactggtgagtacgcc

SEQ ID NO: 125 - DNA, 25 bp, synthetic construct
  source 1..25: mol_type = other DNA
taggacaggtaagagatcaggctga

SEQ ID NO: 126 - DNA, 25 bp, synthetic construct
  source 1..25: mol_type = other DNA
tcaaagcagtaagtagtacatgtaa

SEQ ID NO: 127 - DNA, 25 bp, synthetic construct
  source 1..25: mol_type = other DNA
ctgggcaggtgagtctatgggaccc

SEQ ID NO: 128 - DNA, 12 bp, synthetic construct
  source 1..12: mol_type = other DNA
yyyyyyyncagr

SEQ ID NO: 129 - DNA, 62 bp, synthetic construct
  source 1..62: mol_type = other DNA
ggttcattctcaagcctcagacagtggttcaaagtttttttcttccatttcaggtgtcgtga

SEQ ID NO: 130 - DNA, 59 bp, synthetic construct
  source 1..59: mol_type = other DNA
cagggtggggccacctgccggtaggtgtgcggtaggcttttctccgtcgcaggacgcag

SEQ ID NO: 131 - DNA, 62 bp, synthetic construct
  source 1..62: mol_type = other DNA
tgataggcacctattggtcttactgacatccactttgcctttctctccacaggtgtccactc

SEQ ID NO: 132 - DNA, 62 bp, synthetic construct
  source 1..62: mol_type = other DNA
gcggctttagagcctctgctaaccatgttcatgccttcttctttttcctacagctcctgggc

SEQ ID NO: 133 - DNA, 63 bp, synthetic construct
  source 1..63: mol_type = other DNA
ccaagctaggcccttttgctaatcatgttcatacctcttatcttcctcccacaggtgtccact

SEQ ID NO: 134 - DNA, 59 bp, synthetic construct
  source 1..59: mol_type = other DNA
gtcgactgatcttcagacctggaggaggagatatgagggacaattgatgcatctcgagc

SEQ ID NO: 135 - DNA, 216 bp, synthetic construct
  source 1..216: mol_type = other DNA
aaattggcagtattcatccacaattttaaaagaaaaggggggattggggggtacagtgcaggggaaagaatagtagacataatagcaacagacatacaaactaaagaattacaaaaacaaattacaaaaattcaaaattttcgggtttcacgtgacgcgtctgcagccgaaggaatagaagaagaaggtggagagagagacagagacctgcagacg

SEQ ID NO: 136 - DNA, 42 bp, synthetic construct
  source 1..42: mol_type = other DNA
tggcaggaagaagcggagacagcgacgaagagctcatcagaa

SEQ ID NO: 137 - DNA, 253 bp, synthetic construct
  source 1..253: mol_type = other DNA
ttttggtcgtgaggcactgggcaggaagaagcggagacagcgacgaagagctcatcagaactagtcagactcatcaagcttctctatcaaagcagtaagtagtacatgtaacaaggttacaagacaggtttaaggagaccaatagaaactgggcttgtcgagacagagaagactcttgcgtttctgataggcacctattggtcttactgacatccactttgcctttctctccacaggtgtccactcccagttc

SEQ ID NO: 138 - DNA, 602 bp, synthetic construct
  source 1..602: mol_type = other DNA
ttttggtcgtgaggcactgggcaggaagaagcggagacagcgacgaagagctcatcagaactagtcagactcatcaagcttctctatcaaagcagtaagtagtacatgtaagagtctatgggacccttgatgttttctttccccttcttttctatggttaagttcatgtcataggaaggggagaagtaacagggtacacatattgaccaaatcagggtaattttgcatttgtaattttaaaaaatgctttcttcttttaatatacttttttgtttatcttatttctaatactttccctaatctctttctttcagggcaataatgatacaatgtatcatgcctctttgcaccattctaaagaataacagtgataatttctgggttaaggcaatagcaatatttctgcatataaatatttctgcatataaattgtaactgatgtaagaggtttcatattgctaatagcagctacaatccagctaccattctgcttttattttatggttgggataaggctggattattctgagtccaagctaggcccttttgctaatcatgttcatacctcttatcttcctcccacaggtgtccactcccagttc

SEQ ID NO: 139 - DNA, 834 bp, synthetic construct
  source 1..834: mol_type = other DNA
ttttggtcgtgaggcactgggcaggaagaagcggagacagcgacgaagagctcatcagaactagtcagactcatcaagcttctctatcaaagcagtaagtagtacatgtaagagtctatgggacccttgatgttttctttccccttcttttctatggttaagttcatgtcataggaaggggagaagtaacagggtacacatattgaccaaatcagggtaattttgcatttgtaattttaaaaaatgctttcttcttttaatatacttttttgtttatcttatttctaatactttccctaatctctttctttcagggcaataatgatacaatgtatcatgcctctttgcaccattctaaagaataacagtgataatttctgggttaaggcaatagcaatatttctgcatataaatatttctgcatataaattgtaactgatgtaagaggtttcatattgctaatagcagctacaatccagctaccattctgcttttattttatggttgggataaggctggattattctgagtccaagctaggcccttttgctaatcatgttcatacctcttatcttcctcccacaggtgtccactcccagttcctgcaggcacgtgaaattggcagtattcatccacaattttaaaagaaaaggggggattggggggtacagtgcaggggaaagaatagtagacataatagcaacagacatacaaactaaagaattacaaaaacaaattacaaaaattcaaaattttcgggtttcacgtgacgcgtctgcagccgaaggaatagaagaagaaggtggagagagagacagagacctgcagacgcgt

SEQ ID NO: 140 - DNA, 1263 bp, synthetic construct
  source 1..1263: mol_type = other DNA
gggtctctctggttagaccagatctgagcctgggagctctctggctaactagggaacccactgcttaagcctcaataaagcttgccttgagtgcttcaagtagtgtgtgcccgtctgttgtgtgactctggtaactagagatccctcagacccttttagtcagtgtggaaaatctctagcagtggcgcccgaacagggacttgaaagcgaaagggaaaccagaggagctctctcgacgcaggactcggcttgctgaagcgcgcacggcaagaggcgaggggaaggcaacagataaatatgccttaaaattttgactagcggaggctagaaggagagagacgggtgcgagagcgtcagtattaagcgggggagaattagatcgcgattgggaaaaaattcggttaaggccagggggaaagactcgagcaattttggtcgtgaggcactgggcaggaagaagcggagacagcgacgaagagctcatcagaactagtcagactcatcaagcttctctatcaaagcagtaagtagtacatgtaagagtctatgggacccttgatgttttctttccccttcttttctatggttaagttcatgtcataggaaggggagaagtaacagggtacacatattgaccaaatcagggtaattttgcatttgtaattttaaaaaatgctttcttcttttaatatacttttttgtttatcttatttctaatactttccctaatctctttctttcagggcaataatgatacaatgtatcatgcctctttgcaccattctaaagaataacagtgataatttctgggttaaggcaatagcaatatttctgcatataaatatttctgcatataaattgtaactgatgtaagaggtttcatattgctaatagcagctacaatccagctaccattctgcttttattttatggttgggataaggctggattattctgagtccaagctaggcccttttgctaatcatgttcatacctcttatcttcctcccacaggtgtccactcccagttcctgcaggcacgtgaaattggcagtattcatccacaattttaaaagaaaaggggggattggggggtacagtgcaggggaaagaatagtagacataatagcaacagacatacaaactaaagaattacaaaaacaaattacaaaaattcaaaattttcgggtttcacgtgacgcgtctgcagccgaaggaatagaagaagaaggtggagagagagacagagacctgcagacgcgt

SEQ ID NO: 141 - DNA, 99 bp, synthetic construct
  source 1..99: mol_type = other DNA
accgcgttatccgttcctcgtaggctggtcctggggaacgggtcggcggccggtcggcttctgttttatttttttttttattttttatcttctcctttc

SEQ ID NO: 142 - DNA, 90 bp, synthetic construct
  source 1..90: mol_type = other DNA
cgatccatactgcggaactcctagccgcttgttttgctcgcagcaggtctggagcaaacctcatcgggaccgacaattctgtcgtactct

SEQ ID NO: 143 - DNA, 21 bp, synthetic construct
  source 1..21: mol_type = other DNA; note = HIV vector forward primer
aaagcgaaagggaaaccagag

SEQ ID NO: 144 - DNA, 18 bp, synthetic construct
  source 1..18: mol_type = other DNA; note = HIV vector reverse (GFP) primer
cttgtggccgtttacgtc

SEQ ID NO: 145 - DNA, 18 bp, synthetic construct
  source 1..18: mol_type = other DNA; note = HIV vector reverse (wPRE) primer
agcagcgtatccacatag

SEQ ID NO: 146 - DNA, 30 bp, synthetic construct
  source 1..30: mol_type = other DNA; note = Human Actin cDNA forward primer
tgacggggtcacccacactgtgcccatcta

SEQ ID NO: 147 - DNA, 30 bp, synthetic construct
  source 1..30: mol_type = other DNA; note = Human Actin cDNA reverse primer
ctagaagcatttgcggtggacgatggaggg

SEQ ID NO: 148 - DNA, 57 bp, synthetic construct
  source 1..57: mol_type = other DNA; note = HIV-1 Retrovirus/Hybrid R region loop 1 or synthetic polyA sequence
gggtctctctggttagaccagatctgagcctgggagctctctggctaactagggaac

SEQ ID NO: 149 - DNA, 45 bp, synthetic construct
  source 1..45: mol_type = other DNA; note = RSV Retrovirus/Hybrid R region loop 1 or synthetic polyA sequence
gccattttaccattcaccacattggtgtgcacctgggttgatggc

SEQ ID NO: 150 - DNA, 44 bp, synthetic construct
  source 1..44: mol_type = other DNA; note = MMTV Retrovirus/Hybrid R region loop 1 or synthetic polyA sequence
gcaacagtcctaatattcacgtctcgtgtgtttgtgtctgttcg

SEQ ID NO: 151 - DNA, 43 bp, synthetic construct
  source 1..43: mol_type = other DNA; note = SPA Retrovirus/Hybrid R region loop 1 or synthetic polyA sequence
agatctttattttcattacatctgtgtgttggttttttgtgtg

SEQ ID NO: 152 - DNA, 52 bp, synthetic construct
  source 1..52: mol_type = other DNA; note = 3/1GR-GU1
gggtctctctggttagaccacacattggtgtgcacctggctaactagggaac

SEQ ID NO: 153 - DNA, 57 bp, synthetic construct
  source 1..57: mol_type = other DNA; note = 3/1GR-GU2
gggtctctctggttagaccacacattcgtgtgtttgtgtctgttctaactagggaac

SEQ ID NO: 154 - DNA, 55 bp, synthetic construct
  source 1..55: mol_type = other DNA; note = 3/1GR-GU3
gggtctctctggttagaccacacattggtgtgcacctgggttctaactagggaac

SEQ ID NO: 155 - DNA, 56 bp, synthetic construct
  source 1..56: mol_type = other DNA; note = 3/1GR-GU4
gggtctctctggttagaccacacattggtgtgcacctgtggttctaactagggaac

SEQ ID NO: 156 - DNA, 62 bp, synthetic construct
  source 1..62: mol_type = other DNA; note = 3/1GR-GU5
gggtctctctggttagaccacacatgtctcgtgtgtttgtgtctgttcgctaactagggaac

SEQ ID NO: 157 - DNA, 54 bp, synthetic construct
  source 1..54: mol_type = other DNA; note = 3/1GR-GU6
gggtctctctggttacaccacaatttggtgtgcacctgggtttaactagggaac

SEQ ID NO: 158 - DNA, 62 bp, synthetic construct
  source 1..62: mol_type = other DNA; note = 3/1GR-GU7
gggtctctctggttagaccggcgcagcgtcattggtgtgcacctgggttctaactagggaac

SEQ ID NO: 159 - RNA, 55 nt, synthetic construct
  source 1..55: mol_type = other RNA
gtctctctggttagaccagatctgagcctgggagctctctggctaactagggaac

SEQ ID NO: 160 - RNA, 45 nt, synthetic construct
  source 1..45: mol_type = other RNA
gccattttaccattcaccacattggtgtgcacctgggttgatggc

SEQ ID NO: 161 - RNA, 44 nt, synthetic construct
  source 1..44: mol_type = other RNA
gcaacagtcctaatattcacgtctcgtgtgtttgtgtctgttcg

SEQ ID NO: 162 - RNA, 50 nt, synthetic construct
  source 1..50: mol_type = other RNA
gtctctctggttagaccacacattggtgtgcacctggctaactagggaac

SEQ ID NO: 163 - RNA, 55 nt, synthetic construct
  source 1..55: mol_type = other RNA
gtctctctggttagaccacacattcgtgtgtttgtgtctgttctaactagggaac

SEQ ID NO: 164 - RNA, 53 nt, synthetic construct
  source 1..53: mol_type = other RNA
gtctctctggttagaccacacattggtgtgcacctgggttctaactagggaac

SEQ ID NO: 165 - RNA, 54 nt, synthetic construct
  source 1..54: mol_type = other RNA
gtctctctggttagaccacacattggtgtgcacctgtggttctaactagggaac

SEQ ID NO: 166 - RNA, 60 nt, synthetic construct
  source 1..60: mol_type = other RNA
gtctctctggttagaccacacatgtctcgtgtgtttgtgtctgttcgctaactagggaac

SEQ ID NO: 167 - RNA, 52 nt, synthetic construct
  source 1..52: mol_type = other RNA
gtctctctggttacaccacaatttggtgtgcacctgggtttaactagggaac

SEQ ID NO: 168 - RNA, 60 nt, synthetic construct
  source 1..60: mol_type = other RNA
gtctctctggttagaccggcgcagcgtcattggtgtgcacctgggttctaactagggaac

SEQ ID NO: 169 - RNA, 64 nt, synthetic construct
  source 1..64: mol_type = other RNA
gtctctctggttagacgcacaacacaaaaccgtgtgttggttttttgtgtgctaactagggaac

SEQ ID NO: 170 - DNA, 59 bp, synthetic construct
  source 1..59: mol_type = other DNA; note = HIV-1 R1-59
gggtctctctggttagaccagatctgagcctgggagctctctggctaactagggaaccc

SEQ ID NO: 171 - DNA, 30 bp, synthetic construct
  source 1..30: mol_type = other DNA; note = supA-LTR 3prime (R.1-20)
aataaagggtctctctggttagaccacaca

SEQ ID NO: 172 - DNA, 57 bp, synthetic construct
  source 1..57: mol_type = other DNA; note = 1G 1st ssDNA
cagagagaccaatctggtgtgtaagcacacaaacacagacaagattgatcccttggg

SEQ ID NO: 173 - DNA, 58 bp, synthetic construct
  source 1..58: mol_type = other DNA; note = 2G 1st ssDNA
ccagagagaccaatctggtgtgtaagcacacaaacacagacaagattgatcccttggg

SEQ ID NO: 174 - DNA, 59 bp, synthetic construct
  source 1..59: mol_type = other DNA; note = 3G 1st ssDNA
cccagagagaccaatctggtgtgtaagcacacaaacacagacaagattgatcccttggg

SEQ ID NO: 175 - RNA, 54 nt, synthetic construct
  source 1..54: mol_type = other RNA; note = supA-LTR LV vRNA (3prime end)
aataaagggtctctctggttagaccaaaaaaaaaaaaaaaaaaaaaaaaaaaaa

SEQ ID NO: 176 - DNA, 58 bp, synthetic construct
  source 1..58: mol_type = other DNA; note = HIV-1wt (3G)
cgagccctcagatgctacatataagcagctgctttttgcctgtactgggtctctctgg

SEQ ID NO: 177 - DNA, 57 bp, synthetic construct
  source 1..57: mol_type = other DNA; note = CMV-3G
gtgtacggtgggaggtctatataagcagagctcgtttagtgaaccgggtctctctgg

SEQ ID NO: 178 - DNA, 57 bp, synthetic construct
  source 1..57: mol_type = other DNA; note = CMV-RSV1-1G
gtgtacggtgggaggtctatataagtgcctagctcgatacaataaacgtctctctgg

SEQ ID NO: 179 - DNA, 57 bp, synthetic construct
  source 1..57: mol_type = other DNA; note = CMV-RSV2-1G
gtgtacggtggatattgtatttaagtgcctagctcgatacaataaacgtctctctgg

SEQ ID NO: 180 - DNA, 59 bp, synthetic construct
  source 1..59: mol_type = other DNA; note = RSV-3G
gcatcgcagagatattgtatttaagtgcctagctcgatacaataaacgggtctctctgg

SEQ ID NO: 181 - DNA, 59 bp, synthetic construct
  source 1..59: mol_type = other DNA; note = RSVwt (1G)
gcatcgcagagatattgtatttaagtgcctagctcgatacaataaacgccattttacca

SEQ ID NO: 182 - DNA, 16 bp, synthetic construct
  source 1..16: mol_type = other DNA; note = 1G-R16
gtctctctggttagac

SEQ ID NO: 183 - DNA, 13 bp, synthetic construct
  source 1..13: mol_type = other DNA
aaaagaaaaagaa

SEQ ID NO: 184 - RNA, 23 nt, synthetic construct
  source 1..23: mol_type = other RNA; note = HCMV RNA2.7 ZCCHC14 stem loop
tcctcgtaggctggtcctgggga

SEQ ID NO: 185 - RNA, 20 nt, synthetic construct
  source 1..20: mol_type = other RNA; note = WPRE ZCCHC14
gcccgctgctggacaggggc

SEQ ID NO: 186 - DNA, 50 bp, synthetic construct
  source 1..50: mol_type = other DNA
gtctctctggttagaccacacattggtgtgcacctggctaactagggaac

SEQ ID NO: 187 - DNA, 55 bp, synthetic construct
  source 1..55: mol_type = other DNA
gtctctctggttagaccacacattcgtgtgtttgtgtctgttctaactagggaac

SEQ ID NO: 188 - DNA, 56 bp, synthetic construct
  source 1..56: mol_type = other DNA
gtctctctggttagaccacacacttcgtgtgtttgtgtctgttctaactagggaac

SEQ ID NO: 189 - DNA, 57 bp, synthetic construct
  source 1..57: mol_type = other DNA
gtctctctggttagaccacacacattcgtgtgtttgtgtctgttctaactagggaac

SEQ ID NO: 190 - DNA, 58 bp, synthetic construct
  source 1..58: mol_type = other DNA
gtctctctggttagaccacacacagttcgtgtgtttgtgtctgttctaactagggaac

SEQ ID NO: 191 - DNA, 58 bp, synthetic construct
  source 1..58: mol_type = other DNA
gtctctctggttagaccacacacaattcgtgtgtttgtgtctgttctaactagggaac

SEQ ID NO: 192 - DNA, 59 bp, synthetic construct
  source 1..59: mol_type = other DNA
gtctctctggttagaccacacacagattcgtgtgtttgtgtctgttctaactagggaac

SEQ ID NO: 193 - DNA, 62 bp, synthetic construct
  source 1..62: mol_type = other DNA
gtctctctggttagaccacacattccagattcgtgtgtttgtgtctgttctaactagggaac

SEQ ID NO: 194 - DNA, 52 bp, synthetic construct
  source 1..52: mol_type = other DNA
gtctctctggttagaccacacatggtgtgcacctgggttctaactagggaac

SEQ ID NO: 195 - DNA, 54 bp, synthetic construct
  source 1..54: mol_type = other DNA
gtctctctggttagaccacacattggtgtgcacctgtggttctaactagggaac

SEQ ID NO: 196 - DNA, 60 bp, synthetic construct
  source 1..60: mol_type = other DNA
gtctctctggttagaccacacatgtctcgtgtgtttgtgtctgttcgctaactagggaac

SEQ ID NO: 197 - DNA, 52 bp, synthetic construct
  source 1..52: mol_type = other DNA
gtctctctggttacaccacaatttggtgtgcacctgggtttaactagggaac

SEQ ID NO: 198 - DNA, 60 bp, synthetic construct
  source 1..60: mol_type = other DNA
gtctctctggttagaccggcgcagcgtcattggtgtgcacctgggttctaactagggaac

SEQ ID NO: 199 - DNA, 64 bp, synthetic construct
  source 1..64: mol_type = other DNA
gtctctctggttagacgcacaacacaaaaccgtgtgttggttttttgtgtgctaactagggaac

SEQ ID NO: 200 - DNA, 464 bp, synthetic construct
  source 1..464: mol_type = other DNA
  misc_feature 200..201: note = LV genome/transgene sequences can be inserted between the PBS and the 3prime ppt between nucleotides 200 and 201
gggtctctctggttagaccacacattcgtgtgtttgtgtctgttctaactagggaacccactgcttaagcctcaayaaagcttgccttgagtgcttcaagtagtgtgtgcccgtctgttgtgtgactctggtaactagagatccctcagacccttttagtcagtgtggaaaatctctagcagtggcgcccgaacagggacaaaagaaaaggggggactggaagggctaattcactcccaacgaagacaagatactagttaagatacattgatgagtttggacaaaccacaactagaatgcagtgaaaaaaatgctttatttgtgaaatttgtgatgctattgctttatttgtaaccattataagctgcaataaagggtctctctggttagaccacaagttaacaacaacaattgcattcattttatgtttcaggttcagggggaggtgtgggaggttttttaaa

SEQ ID NO: 201 - DNA, 342 bp, synthetic construct
  source 1..342: mol_type = other DNA
actggaagggctaattcactcccaacgaagacaagatactagttaagatacattgatgagtttggacaaaccacaactagaatgcagtgaaaaaaatgctttatttgtgaaatttgtgatgctattgctttatttgtaaccattataagctgcaataaagggtctctctggttagaccacacattcgtgtgtttgtgtctgttctaactagggaacccactgcttaagcctcaayaaagcttgccttgagtgcttcaagtagtgtgtgcccgtctgttgtgtgactctggtaactagagatccctcagacccttttagtcagtgtggaaaatctctagcagt

SEQ ID NO: 202 - DNA, 33 bp, synthetic construct
  source 1..33: mol_type = other DNA
agcgaacagacacaaacacacgagacatgtgtg

SEQ ID NO: 203 - DNA, 21 bp, synthetic construct
  source 1..21: mol_type = other DNA
acacaaaaaattccaacacac

SEQ ID NO: 204 - DNA, 20 bp, synthetic construct
  source 1..20: mol_type = other DNA
gaacaaacgacccaacaccc

SEQ ID NO: 205 - DNA, 17 bp, synthetic construct
  source 1..17: mol_type = other DNA
ccaacacaccacacaga

SEQ ID NO: 206 - DNA, 26 bp, synthetic construct
  source 1..26: mol_type = other DNA
ccaatgcttatgaataacacaggcga

SEQ ID NO: 207 - DNA, 24 bp, synthetic construct
  source 1..24: mol_type = other DNA
aaaaaccaacacacggttttgtgt

SEQ ID NO: 208 - DNA, 41 bp, synthetic construct
  source 1..41: mol_type = other DNA
taagatacattgatgagtttggacaaaccacaactagaatg

SEQ ID NO: 209 - DNA, 834 bp, synthetic construct
  source 1..834: mol_type = other DNA
  misc_feature 501..502: note = pre-miRNA cassette inserted between nucleotides at position 501 and 502
gaagaagcggagacagcgacgaagagctcaatcagaactagtcagactcaatcaagcttctctatcaaccaggtaagtattacatgtaagagtctatgggacccttgatgttttctttccccttctttttctagatatggttaagttcaatcgattgtcataggaaggggagaagtaacagggtacacatattgaccaaatcagggtaattttgcatttgtaattttaaaaaatgctttcttcttttaatatacttttttgtttatcttatttctaatactttccctaatctctttctttcagggcaataatgagctaagctacaatgtatcatgcctaggcctctttgcaccattctaaagaataacagtgataatttctgggttaaggcaatagcaatatttctgcatataaatatttctgcatataaattgtaactgatgtaagaggtttcatattgctaatagcagctacaatccagctaccattctgcttatgcatttattttatggttggatccgggataaggctggattattctgagtccaagctaggcccttttgctaatcatgttcatacctcttatcttcctcccacaggtgtccactcccagttcctgcaggcacgtgaaattggcagtattcaatccacaattttaaaagaaaaggggggattggggggtacagtgcaggggaaagaatagtagacaataatagcaacagacaatacaaactaaagaattacaaaaacaaattacaaaaattcaaaattttcgggtttcacgtgacgcgtgccgaaggaatagaagaagaaggtggagagagagacagagac

SEQ ID NO: 210 - DNA, 987 bp, synthetic construct
  source 1..987: mol_type = other DNA
  misc_feature 591..592: note = pre-miRNA cassette inserted between nucleotides at position 591 and 592
gaagaagcggagacagcgacgaagagctcaatcagaactagtcagactcaatcaagcttctctatcaaccaggtaagtattacatgtaagagtctatgggacccttgatgttttctttccccttctttttctagatatggttaagttcaatcgattgtcgtggctctcccttagccatccgagtggacgtgcgtcctccttcggatgcccaggtcggaccgcgaggaggtggagatgccatgccgacccataggaaggggagaagtaacagggtacacatattgaccaaatcagggtaattttgcatttgtaattttaaaaaatgctttcttcttttaatatacttttttgtttatcttatttctaatactttccctaatctctttctttcagggcaataatgagctaagctacaatgtatcatgcctaggcctctttgcaccattctaaagaataacagtgataatttctgggttaaggcaatagcaatatttctgcatataaatatttctgcatataaattgtaactgatgtaagaggtttcatattgctaatagcagctacaatccagctaccattctgcttatgcatttattttatggttgcgcgtttcgtcctatttgggactcgtcagctggatgtacccgaagtggaatccaggacgcgcggatccgggataaggctggattattctgagtccaagctaggcccttttgctaatcatgttcatacctcttatcttcctcccacaggtgtccactcccagttcctgcaggcacgtgaaattggcagtattcaatccacaattttaaaagaaaaggggggattggggggtacagtgcaggggaaagaatagtagacaataatagcaacagacaatacaaactaaagaattacaaaaacaaattacaaaaattcaaaattttcgggtttcacgtgacgcgtgccgaaggaatagaagaagaaggtggagagagagacagagac

SEQ ID NO: 211 - DNA, 25 bp, synthetic construct
  source 1..25: mol_type = other DNA
gaagaagcggagacagcgacgaaga

SEQ ID NO: 212 - DNA, 151 bp, synthetic construct
  source 1..151: mol_type = other DNA
aaattggcagtattcaatccacaattttaaaagaaaaggggggattggggggtacagtgcaggggaaagaatagtagacaataatagcaacagacaatacaaactaaagaattacaaaaacaaattacaaaaattcaaaattttcgggttt

SEQ ID NO: 213 - DNA, 148 bp, synthetic construct
  source 1..148: mol_type = other DNA
aaattggcagtattcatccacaattttaaaagaaaaggggggattggggggtacagtgcaggggaaagaatagtagacataatagcaacagacatacaaactaaagaattacaaaaacaaattacaaaaattcaaaattttcgggttt

SEQ ID NO: 214 - DNA, 78 bp, synthetic construct
  source 1..78: mol_type = other DNA
ggctctcccttagccatccgagtggacgtgcgtcctccttcggatgcccaggtcggaccgcgaggaggtggagatgcc

SEQ ID NO: 215 - DNA, 63 bp, synthetic construct
  source 1..63: mol_type = other DNA
gcgcgtttcgtcctatttgggactcgtcagctggatgtacccgaagtggaatccaggacgcgc

SEQ ID NO: 216 - DNA, 19 bp, synthetic construct
  source 1..19: mol_type = other DNA
taaattgtaactgatgtaa

SEQ ID NO: 217 - DNA, 27 bp, synthetic construct
  source 1..27: mol_type = other DNA
caaagtgcttacagtgcaggtagaatt

SEQ ID NO: 218 - DNA, 100 bp, synthetic construct
  source 1..100: mol_type = other DNA
caaagtgcttacagtgcaggtagaatttaaattgtaacaaagtgcttacagtgcaggtagaattctgatgtaacaaagtgcttacagtgcaggtagaatt

SEQ ID NO: 219 - DNA, 27 bp, synthetic construct
  source 1..27: mol_type = other DNA
taaagtgcttatagtgcaggtagaatt

SEQ ID NO: 220 - DNA, 100 bp, synthetic construct
  source 1..100: mol_type = other DNA
taaagtgcttatagtgcaggtagaatttaaattgtaataaagtgcttatagtgcaggtagaattctgatgtaataaagtgcttatagtgcaggtagaatt

SEQ ID NO: 221 - DNA, 27 bp, synthetic construct
  source 1..27: mol_type = other DNA
aaaagtgcttacagtgcaggtagaatt

SEQ ID NO: 222 - DNA, 100 bp, synthetic construct
  source 1..100: mol_type = other DNA
aaaagtgcttacagtgcaggtagaatttaaattgtaaaaaagtgcttacagtgcaggtagaattctgatgtaaaaaagtgcttacagtgcaggtagaatt

SEQ ID NO: 223 - DNA, 147 bp, synthetic construct
  source 1..147: mol_type = other DNA
gatatctcatagattggacttgacacttgatatcgtagagtatggtcaaccttacttgcatagattgggcttgacacttcatctgtggcttcacaagtgtcaagtccaatctatgaaggcactgctgacattgctatcaccatgcat

SEQ ID NO: 224 - DNA, 119 bp, synthetic construct
  source 1..119: mol_type = other DNA
gatatcgtagagtatggtcaaccttacttgcatagattgggcttgacacttcatctgtggcttcacaagtgtcaagtccaatctatgaaggcactgctgacattgctatcaccatgcat

SEQ ID NO: 225 - DNA, 22 bp, synthetic construct
  source 1..22: mol_type = other DNA
tcatagattggacttgacactt

SEQ ID NO: 226 - DNA, 85 bp, synthetic construct
  source 1..85: mol_type = other DNA
gtcaaccttacttgcatagattgggcttgacacttcatctgtggcttcacaagtgtcaagtccaatctatgaaggcactgctgac

SEQ ID NO: 227 - DNA, 10 bp, synthetic construct
  source 1..10: mol_type = other DNA
tcagttcctg

SEQ ID NO: 228 - DNA, 10 bp, synthetic construct
  source 1..10: mol_type = other DNA
gcagttcctg

SEQ ID NO: 229 - DNA, 10 bp, synthetic construct
  source 1..10: mol_type = other DNA
caagttcctg

SEQ ID NO: 230 - DNA, 10 bp, synthetic construct
  source 1..10: mol_type = other DNA
cctgttcctg

SEQ ID NO: 231 - DNA, 10 bp, synthetic construct
  source 1..10: mol_type = other DNA
cctgctcctg

SEQ ID NO: 232 - DNA, 10 bp, synthetic construct
  source 1..10: mol_type = other DNA
cctgtacctg

SEQ ID NO: 233 - DNA, 10 bp, synthetic construct
  source 1..10: mol_type = other DNA
cctgttgctg

SEQ ID NO: 234 - DNA, 10 bp, synthetic construct
  source 1..10: mol_type = other DNA
cctgttcgtg

SEQ ID NO: 235 - DNA, 10 bp, synthetic construct
  source 1..10: mol_type = other DNA
cctgttccag

SEQ ID NO: 236 - DNA, 10 bp, synthetic construct
  source 1..10: mol_type = other DNA
cctgttcctc

SEQ ID NO: 237 - DNA, 10 bp, synthetic construct
  source 1..10: mol_type = other DNA
ccaattcctg

SEQ ID NO: 238 - DNA, 10 bp, synthetic construct
  source 1..10: mol_type = other DNA
gaagctcctg

SEQ ID NO: 239 - DNA, 20 bp, synthetic construct
  source 1..20: mol_type = other DNA; note = Cons/mut5
ccagttcctgccagttccga

SEQ ID NO: 240 - DNA, 141 bp, synthetic construct
  source 1..141: mol_type = other DNA
ccagttcctgccagttcctgccagttcctgccagttcctgactaggtacctcgagcggatcccatcgattgccgtcgccaccgcgttatccgttcctcgtaggctggtcctggggaacgggtcggcggccggtcggcttct

SEQ ID NO: 241 - DNA, 181 bp, synthetic construct
  source 1..181: mol_type = other DNA
ccagttcctgccagttcctgccagttcctgccagttcctgccagttcctgccagttcctgccagttcctgccagttcctgactaggtacctcgagcggatcccatcgattgccgtcgccaccgcgttatccgttcctcgtaggctggtcctggggaacgggtcggcggccggtcggcttct

SEQ ID NO: 242 - DNA, 261 bp, synthetic construct
  source 1..261: mol_type = other DNA
ccagttcctgccagttcctgccagttcctgccagttcctgccagttcctgccagttcctgccagttcctgccagttcctgccagttcctgccagttcctgccagttcctgccagttcctgccagttcctgccagttcctgccagttcctgccagttcctgactaggtacctcgagcggatcccatcgattgccgtcgccaccgcgttatccgttcctcgtaggctggtcctggggaacgggtcggcggccggtcggcttct

SEQ ID NO: 243 - DNA, 10 bp, synthetic construct
  source 1..10: mol_type = other DNA
bmwrhwssws

SEQ ID NO: 244 - DNA, 66 bp, synthetic construct
  source 1..66: mol_type = other DNA
gggtctctctggttagacgcacaacacaaaaccgtgtgttggttttttgtgtgctaactagggaac

SEQ ID NO: 245 - DNA, 18 bp, synthetic construct
  source 1..18: mol_type = other DNA; note = 3G-R18
gggtctctctggttagac

SEQ ID NO: 246 - DNA, 10 bp, synthetic construct
  source 1..10: mol_type = other DNA
ccagttccga

SEQ ID NO: 247 - DNA, 166 bp, synthetic construct
  source 1..166: mol_type = other DNA
ttagccagagagctcccaggctcagatctggtctaaccagagagaccctttattgcagcttataatggttacaaataaagcaatagcatcacaaatttcacaaataaagcatttttttcactgactagtatcttgtcttcgttgggagtgaattagcccttccagt

SEQ ID NO: 248 - DNA, 154 bp, synthetic construct
  source 1..154: mol_type = other DNA
ttagccagagagctcccaggctcagatctggtctaaccagagagaccctttattgcagcttataatggttacagcaatagcatcacaaatttcacagcatttttttcactgactagtatcttgtcttcgttgggagtgaattagcccttccagt

SEQ ID NO: 249 - DNA, 166 bp, synthetic construct
  source 1..166: mol_type = other DNA
ttagaacagacacaaacacacgaatgtgtggtctaaccagagagaccctttattgcagcttataatggttacaaataaagcaatagcatcacaaatttcacaaataaagcatttttttcactgactagtatcttgtcttcgttgggagtgaattagcccttccagt

SEQ ID NO: 250 - DNA, 154 bp, synthetic construct
  source 1..154: mol_type = other DNA
ttagaacagacacaaacacacgaatgtgtggtctaaccagagagaccctttattgcagcttataatggttacagcaatagcatcacaaatttcacagcatttttttcactgactagtatcttgtcttcgttgggagtgaattagcccttccagt

SEQ ID NO: 251 - DNA, 206 bp, synthetic construct
  source 1..206: mol_type = other DNA
ttagccagagagctcccaggctcagatctggtctaaccagagagaccctttattgcagcttataatggttacaataaagcaatagcatcacaaatttcacaaataaagcatttttttcactgcattctagttgtggtttgtccaaactcatcaatgtatcttaactagtatcttgtcttcgttgggagtgaattagcccttccagt

SEQ ID NO: 252 - DNA, 206 bp, synthetic construct
  source 1..206: mol_type = other DNA
ttagaacagacacaaacacacgaatgtgtggtctaaccagagagaccctttattgcagcttataatggttacaataaagcaatagcatcacaaatttcacaaataaagcatttttttcactgcattctagttgtggtttgtccaaactcatcaatgtatcttaactagtatcttgtcttcgttgggagtgaattagcccttccagt

SEQ ID NO: 253 - DNA, 198 bp, synthetic construct
  source 1..198: mol_type = other DNA
ttagccagagagctcccaggctcagatctggtctaaccagagagaccctttattgcagcttataatggttacaataaagcaatagcatcacaaatttcacaaataaagcatttttttcactgcacacatgtctcgtgtgtttgtgtctgttcgctactagtatcttgtcttcgttgggagtgaattagcccttccagt

SEQ ID NO: 254 - DNA, 198 bp, synthetic construct
  source 1..198: mol_type = other DNA
ttagaacagacacaaacacacgaatgtgtggtctaaccagagagaccctttattgcagcttataatggttacaataaagcaatagcatcacaaatttcacaaataaagcatttttttcactgcacacatgtctcgtgtgtttgtgtctgttcgctactagtatcttgtcttcgttgggagtgaattagcccttccagt

SEQ ID NO: 255 - DNA, 186 bp, synthetic construct
  source 1..186: mol_type = other DNA
ttagccagagagctcccaggctcagatctggtctaaccagagagaccctttattgcagcttataatggttacaataaagcaatagcatcacaaatttcacaaataaagcatttttttcactggtgtgttggaattttttgtgtactagtatcttgtcttcgttgggagtgaattagcccttccagt

SEQ ID NO: 256 - DNA, 186 bp, synthetic construct
  source 1..186: mol_type = other DNA
ttagaacagacacaaacacacgaatgtgtggtctaaccagagagaccctttattgcagcttataatggttacaataaagcaatagcatcacaaatttcacaaataaagcatttttttcactggtgtgttggaattttttgtgtactagtatcttgtcttcgttgggagtgaattagcccttccagt

SEQ ID NO: 257 - DNA, 185 bp, synthetic construct
  source 1..185: mol_type = other DNA
ttagccagagagctcccaggctcagatctggtctaaccagagagaccctttattgcagcttataatggttacaataaagcaatagcatcacaaatttcacaaataaagcatttttttcactggggtgttgggtcgtttgttcactagtatcttgtcttcgttgggagtgaattagcccttccagt

SEQ ID NO: 258 - DNA, 185 bp, synthetic construct
  source 1..185: mol_type = other DNA
ttagaacagacacaaacacacgaatgtgtggtctaaccagagagaccctttattgcagcttataatggttacaataaagcaatagcatcacaaatttcacaaataaagcatttttttcactggggtgttgggtcgtttgttcactagtatcttgtcttcgttgggagtgaattagcccttccagt

SEQ ID NO: 259 - DNA, 182 bp, synthetic construct
  source 1..182: mol_type = other DNA
ttagccagagagctcccaggctcagatctggtctaaccagagagaccctttattgcagcttataatggttacaataaagcaatagcatcacaaatttcacaaataaagcatttttttcactgtctgtgtggtgtgttggactagtatcttgtcttcgttgggagtgaattagcccttccagt

SEQ ID NO: 260 - DNA, 182 bp, synthetic construct
  source 1..182: mol_type = other DNA
ttagaacagacacaaacacacgaatgtgtggtctaaccagagagaccctttattgcagcttataatggttacaataaagcaatagcatcacaaatttcacaaataaagcatttttttcactgtctgtgtggtgtgttggactagtatcttgtcttcgttgggagtgaattagcccttccagt

SEQ ID NO: 261 - DNA, 191 bp, synthetic construct
  source 1..191: mol_type = other DNA
ttagccagagagctcccaggctcagatctggtctaaccagagagaccctttattgcagcttataatggttacaataaagcaatagcatcacaaatttcacaaataaagcatttttttcactgtcgcctgtgttattcataagcattggactagtatcttgtcttcgttgggagtgaattagcccttccagt

SEQ ID NO: 262 - DNA, 191 bp, synthetic construct
  source 1..191: mol_type = other DNA
ttagaacagacacaaacacacgaatgtgtggtctaaccagagagaccctttattgcagcttataatggttacaataaagcaatagcatcacaaatttcacaaataaagcatttttttcactgtcgcctgtgttattcataagcattggactagtatcttgtcttcgttgggagtgaattagcccttccagt

SEQ ID NO: 263 - DNA, 189 bp, synthetic construct
  source 1..189: mol_type = other DNA
ttagccagagagctcccaggctcagatctggtctaaccagagagaccctttattgcagcttataatggttacaataaagcaatagcatcacaaatttcacaaataaagcatttttttcactgacacaaaaccgtgtgttggtttttactagtatcttgtcttcgttgggagtgaattagcccttccagt

SEQ ID NO: 264 - DNA, 189 bp, synthetic construct
  source 1..189: mol_type = other DNA
ttagaacagacacaaacacacgaatgtgtggtctaaccagagagaccctttattgcagcttataatggttacaataaagcaatagcatcacaaatttcacaaataaagcatttttttcactgacacaaaaccgtgtgttggtttttactagtatcttgtcttcgttgggagtgaattagcccttccagt